European Patent Specification EP 4 003 515 B1, published October 22, 2025. Title: KLF INDUCED CARDIOMYOGENESIS. Applicant: Victor Chang Cardiac Research Institute National Cerebral and Cardiovascular Center. The sequence listing filed with the application follows.

SEQUENCE LISTING (11 sequences)

SEQ ID NO: 1 - protein, 362 aa, Homo sapiens
MATAETALPSISTLTALGPFPDTQDDFLKWWRSEEAQDMGPGPPDPTEPPLHVKSEDQPGEEEDDERGADATWDLDLLLTNFSGPEPGGAPQTCALAPSEASGAQYPPPPETLGAYAGGPGLVAGLLGSEDHSGWVRPALRARAPDAFVGPALAPAPAPEPKALALQPVYPGPGAGSSGGYFPRTGLSVPAASGAPYGLLSGYPAMYPAPQYQGHFQLFRGLQGPAPGPATSPSFLSCLGPGTVGTGLGGTAEDPGVIAETAPSKRGRRSWARKRQAAHTCAHPGCGKSYTKSSHLKAHLRTHTGEKPYACTWEGCGWRFARSDELTRHYRKHTGQRPFRCQLCPRAFSRSDHLALHMKRHL

SEQ ID NO: 2 - DNA, 1645 bp, Homo sapiens
tcagagttcacgaggcagccgaggaagaggaggcttgaggcccagggtgggcaccagccagccatggccacagccgagaccgccttgccctccatcagcacactgaccgccctgggccccttcccggacacacaggatgacttcctcaagtggtggcgctccgaagaggcgcaggacatgggcccgggtcctcctgaccccacggagccgcccctccacgtgaagtctgaggaccagcccggggaggaagaggacgatgagaggggcgcggacgccacctgggacctggatctcctcctcaccaacttctcgggcccggagcccggtggcgcgccccagacctgcgctctggcgcccagcgaggcctccggggcgcaatatccgccgccgcccgagactctgggcgcatatgctggcggcccggggctggtggctgggcttttgggttcggaggatcactcgggttgggtgcgccctgccctgcgagcccgggctcccgacgccttcgtgggcccagccctggctccagccccggcccccgagcccaaggcgctggcgctgcaaccggtgtacccggggcccggcgccggctcctcgggtggctacttcccgcggaccgggctttcagtgcctgcggcgtcgggcgccccctacgggctactgtccgggtaccccgcgatgtacccggcgcctcagtaccaagggcacttccagctcttccgcgggctccagggacccgcgcccggtcccgccacgtccccctccttcctgagttgtttgggacccgggacggtgggcactggactcggggggactgcagaggatccaggtgtgatagccgagaccgcgccatccaagcgaggccgacgttcgtgggcgcgcaagaggcaggcagcgcacacgtgcgcgcacccgggttgcggcaagagctacaccaagagctcccacctgaaggcgcatctgcgcacgcacacaggggagaagccatacgcctgcacgtgggaaggctgcggctggagattcgcgcgctcggacgagctgacccgccactaccggaaacacacggggcagcgccccttccgctgccagctctgcccacgtgctttttcgcgctctgaccacctggccttgcacatgaagcgccacctttgagccctgccctggcacttggactctcctagtgactggggatgggacaagaagcctgtttggtggtctcttcacacggacgcgcgtgacacaatgctgggtggttttcccacgaatggaccctctcctggactcgcgttcccaaagatccacccaaatatcaaacacggacccatagacagccctgggggagcctcttacggaaaatccgacaagccttcagccacagggagccacacagagatgtccaaactgtcgtgcaaacccagtgagacagaccgccaaataaacggactcagtggacactcagaccagctcccagatggccctggacagcaggagagggtgtgggatgaggcttcccagagaccctgggtctagaaagcggctcctgaaggtcccttattgtggctgatattaactgtcaatggttatgggtcctataaaaatgcccctcccagataaaaaaaaaaaaaaaaaaaaaaaaaaaaaaaaa

SEQ ID NO: 3 - DNA, 1089 bp, Homo sapiens
atggccacagccgagaccgccttgccctccatcagcacactgaccgccctgggccccttcccggacacacaggatgacttcctcaagtggtggcgctccgaagaggcgcaggacatgggcccgggtcctcctgaccccacggagccgcccctccacgtgaagtctgaggaccagcccggggaggaagaggacgatgagaggggcgcggacgccacctgggacctggatctcctcctcaccaacttctcgggcccggagcccggtggcgcgccccagacctgcgctctggcgcccagcgaggcctccggggcgcaatatccgccgccgcccgagactctgggcgcatatgctggcggcccggggctggtggctgggcttttgggttcggaggatcactcgggttgggtgcgccctgccctgcgagcccgggctcccgacgccttcgtgggcccagccctggctccagccccggcccccgagcccaaggcgctggcgctgcaaccggtgtacccggggcccggcgccggctcctcgggtggctacttcccgcggaccgggctttcagtgcctgcggcgtcgggcgccccctacgggctactgtccgggtaccccgcgatgtacccggcgcctcagtaccaagggcacttccagctcttccgcgggctccagggacccgcgcccggtcccgccacgtccccctccttcctgagttgtttgggacccgggacggtgggcactggactcggggggactgcagaggatccaggtgtgatagccgagaccgcgccatccaagcgaggccgacgttcgtgggcgcgcaagaggcaggcagcgcacacgtgcgcgcacccgggttgcggcaagagctacaccaagagctcccacctgaaggcgcatctgcgcacgcacacaggggagaagccatacgcctgcacgtgggaaggctgcggctggagattcgcgcgctcggacgagctgacccgccactaccggaaacacacggggcagcgccccttccgctgccagctctgcccacgtgctttttcgcgctctgaccacctggccttgcacatgaagcgccacctttga

SEQ ID NO: 4 - DNA, 1476 bp, Mus musculus
agaagagagagaggaggcctgaggtccagggtggacaccagccagccatggcctcagctgagactgtcttaccctccatcagtacactcaccaccctgggacagttcctggacacccaggaggacttcctcaagtggtggcggtctgaggagacgcaggatttggggccggggcccccgaatcccacggggccgtcccatcacgtgagtctgaaatcggaggacccttccggagaggacgatgagagggacgtgacctgtgcgtgggacccggatcttttccttacaaactttccaggttccgagtctcccggcacttcccggacctgtgccctggcgcccagcgtggggccagtggcacagttcgagccgcctgagtctctgggcgcctatgcgggtggcccagggttggtgactgggcctttgggctccgaggagcacacaagctgggcgcacccgactccgagacccccagcccctgaacccttcgtggcccctgccctggccccgggactcgctcccaaggctcagccctcgtactccgactcgcgagcgggctccgtagggggcttcttcccgcgggcggggcttgcggtgcccgcagctccaggcgccccctatgggctgctgtcgggataccccgcgctgtaccccgcgccacagtaccaaggccacttccagctctttcgcgggctcgcggcgccttctgctggtcccacggcgcccccttccttcttgaattgtctgggacctgggactgtggccacagaactcggggccactgcgatcgccggagacgcaggcttgtccccgggaactgcgccgcccaaacgcagccggcgaactttggcacctaagaggcaggcggcacatacgtgcgggcacgaaggctgcgggaagagctacaccaagagctcgcacctcaaggcgcacctgcgcacgcacacgggagagaagccttatgcctgctcctgggacggctgtgactggaggttcgctcgctcagacgaactgacgcgccactaccggaagcacactggacatcgtcccttctgctgtggcctctgcccacgtgctttttcacgctctgaccacttagctctgcacatgaagcgtcacctctgagtgatcctgcacaaggactggggatgaaataagagtggatccaaggaccgtatcccaaaagatgggccattatatagtcctacccagatcaaaaactgaccagaagaccatacaaaggagccttcaggacaaacctcacatgtcctcagggagccccacacatggccccacagacccagcaatatagaccaccagataaatcaactcaaatggacccctagaccagaggagtgaccctgtgtcctggacgcagatggactggggtgagatttcctaagatctagaagggagcttcacactgtgcccatctgctaggattgttgtcgttactataaaaatttcccatataaaa

SEQ ID NO: 5 - DNA, 1077 bp, Mus musculus
atggcctcagctgagactgtcttaccctccatcagtacactcaccaccctgggacagttcctggacacccaggaggacttcctcaagtggtggcggtctgaggagacgcaggatttggggccggggcccccgaatcccacggggccgtcccatcacgtgagtctgaaatcggaggacccttccggagaggacgatgagagggacgtgacctgtgcgtgggacccggatcttttccttacaaactttccaggttccgagtctcccggcacttcccggacctgtgccctggcgcccagcgtggggccagtggcacagttcgagccgcctgagtctctgggcgcctatgcgggtggcccagggttggtgactgggcctttgggctccgaggagcacacaagctgggcgcacccgactccgagacccccagcccctgaacccttcgtggcccctgccctggccccgggactcgctcccaaggctcagccctcgtactccgactcgcgagcgggctccgtagggggcttcttcccgcgggcggggcttgcggtgcccgcagctccaggcgccccctatgggctgctgtcgggataccccgcgctgtaccccgcgccacagtaccaaggccacttccagctctttcgcgggctcgcggcgccttctgctggtcccacggcgcccccttccttcttgaattgtctgggacctgggactgtggccacagaactcggggccactgcgatcgccggagacgcaggcttgtccccgggaactgcgccgcccaaacgcagccggcgaactttggcacctaagaggcaggcggcacatacgtgcgggcacgaaggctgcgggaagagctacaccaagagctcgcacctcaaggcgcacctgcgcacgcacacgggagagaagccttatgcctgctcctgggacggctgtgactggaggttcgctcgctcagacgaactgacgcgccactaccggaagcacactggacatcgtcccttctgctgtggcctctgcccacgtgctttttcacgctctgaccacttagctctgcacatgaagcgtcacctctga

SEQ ID NO: 6 - protein, 363 aa, Danio rerio
MALPCLLPSISTFANQKEKLWEDRWKIEEHKPLNASCPPLNVALNTDTCRGRKDDEDLSNYLDLEFILANTTGPLEAGAEFISHSEPCGMYSTAVYSSPEAPPPYGLMAELLRSDVDSTYDTTVQGRFLLNSSGFPRQEFPEIKVEPPMDGYGPVIGMVPQTCQKIKQEGNVSCMMSFEQPRLAVSPQATGNMTPPLSPDDSHLRQTTYTQSYHHSPPAYPQVPMQFTAPHQFAMYEEAMGMQPSMQRALLTPPSSPLELMESKPKRGRRTWPRKRMATHTCTYAGCGKTYTKSSHLKAHHRTHTGEKPYHCNWEGCGWKFARSDELTRHFRKHTGHRPFQCHLCERAFSRSDHLALHMKRHL

SEQ ID NO: 7 - DNA, 3573 bp, Danio rerio
ggcacgaggcgcactgtgccttatatatagactatctttgggaactctgaacgcggtttccaccgcgcacacaattggtctaggagccgtatttattaagtaggaggcgctccagccgggcaaactttgttcatgactgtggaagttcactcgaggaaaaagcgcgcagacgtttgacatctcttcaggagcaagtgcattaatactgaatacacaccgagcacgcgtggacatggctttaccttgccttttgccttcgatttcaacgtttgcaaaccagaaggagaagctctgggaggatagatggaagattgaggagcacaaaccactgaacgccagctgccctccgctcaacgtggcactgaacacagacacttgtcgaggccgcaaggatgacgaggatctcagcaattatttagacctggagtttatcctggccaacaccacgggccctctggaggccggagccgagttcatctcccactccgagccatgcggcatgtactccactgcagtttactcatctccagaagcacctccaccatacggcctcatggcagagctcctgcgatctgatgtagactccacgtatgacaccacagtgcaggggagattcctgctcaactccagcggcttccccagacaggagtttcctgaaatcaaagtggagccgccgatggatggctacggtccggtgataggcatggtgccacaaacctgccaaaaaatcaagcaggaaggcaacgtttcatgcatgatgtctttcgagcagcccagactagcagtttctccgcaggccaccgggaatatgactcctccgctgagtcctgacgactcccacctccgtcaaacgacatatacacagagctaccatcactctcctccggcgtatccgcaggtgccaatgcagttcacagcgccacaccagtttgccatgtatgaggaggcaatggggatgcaacccagcatgcagcgggctcttctcacccctccgtcctctccgttagagctaatggagtccaaacccaagcgagggcgacgcacctggccgaggaagcgcatggcgacacatacatgcacgtacgccggctgcgggaagacgtacaccaaaagctcccatttaaaagcgcatcaccgcactcacaccggtgaaaaaccataccactgcaactgggagggatgcggatggaagttcgcccgttctgacgagctgacgcgtcacttccgtaaacacacgggccaccggccgttccagtgccacctgtgtgaacgtgccttctcccgctccgaccacctggcgctgcacatgaagagacacctgtgagggccggatccaccacaactgccttatttaatgactcttattatatatatatatcatcatacttttataacaaagtagctggtactacatagatcacgcagagctctttttaaggcctttttttggggttaaaaagcatcctgaaaggctggtcctacgaatcggtgtccaatccggagactgttatgttgaattaacgatgccacaacgagtgcaaagcctgacgactagcaaaccaaagtggaaaatgcacaacgatgttgacaatgttttgctcgaaactgccatgcaacaaatgtgtttcatttttaccagggctgggaggataaaatcattattgtgaatcaagaaatgattcctacattttctgaatgcattgcgatttccttttgaatcgatttgaagcttagtttttaccaccagagggcactgtatgctttacacatacaatttaaatgtaaaacaattattaatacatacatttgtacataaactagcctagacctctgttaaaagttaacctatagtgcgtctgctgttaaaaactagcctagagcgccctctagtgttaaaaactagcctagagtactgtctggtgtttacaaactagtctagagcttcatctactgttcaaacctagcctagacctctgttaaagattaacctatagtgcttctgctgttaaaaactagcatagagctgcctctggtgttaaaaactagcctagagtgtcatctgctgtttgaaaactagcctagagtgcattcttctgctcaaaactagccttgacctctgttaaaattagcctatagtgcgtctgctgttaaaaactagcctagagcgccatctggtgttaaaaactagcctagagcgccctctgctgctcaaaactaacctaaacctctgttaaaaattagcctatatagtgtctggtgttaaacactagtctagactgccctctgatgttaaaaaaactagcctagagtgccttttgttgcttaaaactagcctagacctcagtttaaaaattagcctacagtgcatctgctgataaaaactagcctagagcgctctcaggtgttaaaaactagcctagagtgccgtctgcttctcaaaaactagcctagagttgattcctttgctcaaaactagcctagacctctgttaaaaaattagcctatagtgcgtctgctgttacaaactagcccagaacatcatctggtgttaataactagcctagagcgccatctgctgctcagaactagcctagacctctgttaaaaattagcctttagtgcgtctccggttaaaaactagcctagagcgccctctagtgttaaaaactagtctagagcgccctctgctgcacaaaattagcctaaacctctgttaaaattagacaagagtgcgtttgctggtaaaaactagcatagagcaccctctggtgttaaaatctagcctagagcacactgtggtgttaaaaactagccaagagcgccatttgcagttcaaaactagcctagattgctgttaaacattagtctagattccatatgctgttataaactcacctagagcgccatctgctgtcaaaaaacccacctagagcgccatctgctgttaaaaacggatcttagaattgattccatagagaatcgggacgcagttaaaaatctaacaatcgattcatgaataacaatacaatgatttatcaattccagccctaattttttacatatttctttccaaatgttggtaacgctttacaataatgctgcatttagtaaatgcattgagcaaaaaaaagtgtgtaatttaggtgcattggatcacaccaacagatgcaacttttgtaagtgttaaagggacggctcactccaaaaatgaagatgacctccattgactttaatagtaattgtttttttatcctatggaagtcagtggagaccatcaagtagcattcttcaaaatatcttctgtagtgtttaacagatgaaaagagtgagtgaatgatgacagatctaattccttgtgtgaactatccctttaacgcatgttccctattgtaaaacattcctcaaacggcggcacattcagtgtcctcttgttcaatagcaccggatgcgctgggtcttgaagtcctgggtctttttttatatgattgtgtacatacattttatattgtaagtactgtatttattgtaaatattaaactaaatttgaatataaaaaaaaaaaaaaaaaaaaaa

SEQ ID NO: 8 - DNA, 1092 bp, Danio rerio
atggctttaccttgccttttgccttcgatttcaacgtttgcaaaccagaaggagaagctctgggaggatagatggaagattgaggagcacaaaccactgaacgccagctgccctccgctcaacgtggcactgaacacagacacttgtcgaggccgcaaggatgacgaggatctcagcaattatttagacctggagtttatcctggccaacaccacgggccctctggaggccggagccgagttcatctcccactccgagccatgcggcatgtactccactgcagtttactcatctccagaagcacctccaccatacggcctcatggcagagctcctgcgatctgatgtagactccacgtatgacaccacagtgcaggggagattcctgctcaactccagcggcttccccagacaggagtttcctgaaatcaaagtggagccgccgatggatggctacggtccggtgataggcatggtgccacaaacctgccaaaaaatcaagcaggaaggcaacgtttcatgcatgatgtctttcgagcagcccagactagcagtttctccgcaggccaccgggaatatgactcctccgctgagtcctgacgactcccacctccgtcaaacgacatatacacagagctaccatcactctcctccggcgtatccgcaggtgccaatgcagttcacagcgccacaccagtttgccatgtatgaggaggcaatggggatgcaacccagcatgcagcgggctcttctcacccctccgtcctctccgttagagctaatggagtccaaacccaagcgagggcgacgcacctggccgaggaagcgcatggcgacacatacatgcacgtacgccggctgcgggaagacgtacaccaaaagctcccatttaaaagcgcatcaccgcactcacaccggtgaaaaaccataccactgcaactgggagggatgcggatggaagttcgcccgttctgacgagctgacgcgtcacttccgtaaacacacgggccaccggccgttccagtgccacctgtgtgaacgtgccttctcccgctccgaccacctggcgctgcacatgaagagacacctgtga

SEQ ID NO: 9 - DNA, 2532 bp, Danio rerio
ggcacgaggataaagtaacctttaatggcactgtgaagttttatgtaaatatatttgactttaacactaaattctgggttcttaccctttgtgtattgcacatgtaaataaatacaattctggacaaatatcaaacactctatttggagacaattgtttgtgtaataaatgctgaaagggcaccaaacggatggctgtgactcaagccgtactgccttcattttcaaacttctgcaccaactccgaaaacatgaagtttgaaaaaggctttctggatctggactccaaggatctgcaccaaagcccagccagctacaaaccttcccagttcctgactgatgagcaccaggacgacagcgagggatgctgggacatggagttcctactgtctgactgggccagtatgtcacctgaacggtccaactctcaaaactacactccccagcggccgaccctacaggaccagcttcacagtccagatctttatcaggagctgaacgcaccaaaaccaaacagacatcaagtgtgcgttgcaagttccctagctgagctgcttcctcctgaagcaaccttaagttcctccctgcctcctgacctccagtttaattgtggatttctagatcaacaagctgccaaatcatattcccaggcagaaaacccccagcagttcagtgctttccctgtcacaagtaatgtaaacagagacagcagcatgggaaaaatggggaagtcctgggatttcggacattactatcagcctgcgcctctgatatccttcccagactccaaatttgtccaaacgcaggggatcacaatggaaacagtggtctttcctccgcatcatcactacaacttcatcccgagctactcgcatcccagactctaccagcagcaggcaaactacgtccacaggccgccgccgcagagccactttccctccacacagagcatggtgcccgactccacagtgccgcctgcaggccttgagagcaagcgcatccgcagagggctggtcaagaggaaagccacggtgcacagctgtgaatatccaggctgccagaagacatacaccaagagctctcatctcaaagcacacctccgtacacacacaggtgaaaagccgtatcactgcacatgggatggctgcgggtggaagttcgcccgttcagacgagctgacgagacacttccgaaaacacaccggacagaagccgtatgagtgtctgctgtgccacagagccttcagcaggtccgaccacctggcgttacacatgaagagacacgtgtgaggaaaaacactaacaaaacacaacaaaccacatgagcttcatccatttcaaaggcttgcgaggacctgtgttcagctggagagatgctggacgctgtttatgcatgataaagaaagtatagaagcactattatatacacatacaatcagtgttgggggtaacgtgttacaagtaatgcagatattactttttgaagtaaagagtaaagtgatgcagtacttttaaaaatgaatgtaatgcaagttactttttagtttaattaacccagatagcacacatacacttgaagtcagaattattagtccccctgtatacttttctcccaatttctttttaacagagaaaaaatttatttctgaacacaatagctttaataactcatttctaataactgatttattttatttactttgccatggtgataataaataatattttactagctattttttcaagacacttctatacaacttaaagtgacatttaaaggcttaactaggtttattaggcaattcattgtataacagtggtttgttctgtagacaataaaaaaatgcttaaggaggctaataatattgaccttaaaatgtctttaaaaaattggaaactgcttttattttagcggaaataaaacaaataagactttctctagaagaaataaatattataagaaatactgtgaaaagttccttgctctgttaaacatcatttgggaaaaataaaaaaaaatgtaacaaataaataaaataaaataaattacaggagggcgaatacttttgacttcaactatacgtcgaggaaaagtcaatgaaagatcgtaacatctacagcatcgcattcgatcaaacatttgtattttaatgagccgtcttctttacctctatacactgtctatgaatcttcaactcctgaaattatgcgatggcaagctctggtaaaaagacgcaacaacttcatcttgaatagctttaaaaaattcattgttgaattaaaattgacattttgaaaagtggattgtctcactgggactgactacttaatgcataggaaaaaagtacaaaagtagcaaacatgttgctttaaatttgcattattctgtatatacagcatgtatagctcaaaagatcactttattctaaacaacttttagatgtgtgtgtgtgtttttttaaagctaaacaaaagttatagagagtgttgttagttgcaaagctcgtcatataaaaaaaaaaaaaaaaaaaaaa

SEQ ID NO: 10 - DNA, 1098 bp, Danio rerio
atggctgtgactcaagccgtactgccttcattttcaaacttctgcaccaactccgaaaacatgaagtttgaaaaaggctttctggatctggactccaaggatctgcaccaaagcccagccagctacaaaccttcccagttcctgactgatgagcaccaggacgacagcgagggatgctgggacatggagttcctactgtctgactgggccagtatgtcacctgaacggtccaactctcaaaactacactccccagcggccgaccctacaggaccagcttcacagtccagatctttatcaggagctgaacgcaccaaaaccaaacagacatcaagtgtgcgttgcaagttccctagctgagctgcttcctcctgaagcaaccttaagttcctccctgcctcctgacctccagtttaattgtggatttctagatcaacaagctgccaaatcatattcccaggcagaaaacccccagcagttcagtgctttccctgtcacaagtaatgtaaacagagacagcagcatgggaaaaatggggaagtcctgggatttcggacattactatcagcctgcgcctctgatatccttcccagactccaaatttgtccaaacgcaggggatcacaatggaaacagtggtctttcctccgcatcatcactacaacttcatcccgagctactcgcatcccagactctaccagcagcaggcaaactacgtccacaggccgccgccgcagagccactttccctccacacagagcatggtgcccgactccacagtgccgcctgcaggccttgagagcaagcgcatccgcagagggctggtcaagaggaaagccacggtgcacagctgtgaatatccaggctgccagaagacatacaccaagagctctcatctcaaagcacacctccgtacacacacaggtgaaaagccgtatcactgcacatgggatggctgcgggtggaagttcgcccgttcagacgagctgacgagacacttccgaaaacacaccggacagaagccgtatgagtgtctgctgtgccacagagccttcagcaggtccgaccacctggcgttacacatgaagagacacgtgtga

SEQ ID NO: 11 - protein, 365 aa, Danio rerio
MAVTQAVLPSFSNFCTNSENMKFEKGFLDLDSKDLHQSPASYKPSQFLTDEHQDDSEGCWDMEFLLSDWASMSPERSNSQNYTPQRPTLQDQLHSPDLYQELNAPKPNRHQVCVASSLAELLPPEATLSSSLPPDLQFNCGFLDQQAAKSYSQAENPQQFSAFPVTSNVNRDSSMGKMGKSWDFGHYYQPAPLISFPDSKFVQTQGITMETVVFPPHHHYNFIPSYSHPRLYQQQANYVHRPPPQSHFPSTQSMVPDSTVPPAGLESKRIRRGLVKRKATVHSCEYPGCQKTYTKSSHLKAHLRTHTGEKPYHCTWDGCGWKFARSDELTRHFRKHTGQKPYECLLCHRAFSRSDHLALHMKRHV